European Patent Application EP 4 556 605 A1, published May 21, 2025. Title: DNA Methylation Library Construction Method and Library Obtained with Same, DNA Hybridization and Capture Method and Kits. Applicant: BOE Technology Group Co., Ltd. The sequence listing filed with the application follows.

SEQUENCE LISTING (4 sequences)

SEQ ID NO: 1 - DNA, 33 bp, synthetic construct
  source 1..33: mol_type = other DNA
acactctttccctacacgacgctcttccgatct

SEQ ID NO: 2 - DNA, 40 bp, synthetic construct
  source 1..40: mol_type = other DNA
nnnnnnnagatcggaagagcgtcgtgtagggaaagagtgt

SEQ ID NO: 3 - DNA, 32 bp, synthetic construct
  source 1..32: mol_type = other DNA
agatcggaagagcacacgtctgaactccagtc

SEQ ID NO: 4 - DNA, 39 bp, synthetic construct
  source 1..39: mol_type = other DNA
gactggagttcagacgtgtgctcttccgatctnnnnnnn